European Patent Specification EP 3 468 375 B1, published September 9, 2026. Title: Fermented milk product with a redued content of lactose. Applicant: Chr. Hansen A/S. The sequence listing filed with the application follows.

SEQUENCE LISTING (4 sequences)

SEQ ID NO: 1 - protein, 1931 aa, Bifidobacterium bifidum
MKKPLGKIVASTALLISVAFSSSIASAAVEDATRSDSTTQMSSTPEVAYSSAVDSKQNRTSDFDANWKFMLSDSVQAQDPAFDDSAWQQVDLPHDYSITQKYSQSNEAESAYLPGGTGWYRKSFTIDRDLAGKRIAINFDGVYMNATVWFNGVKLGTHPYGYSPFSFDLTGNAKFGGENTIVVKVENRLPSSRWYSGSGIYRDVTLTVTDGVHVGNNGVAIKTPSLATQNGGDVTMNLTTKVANDTEAAANITLKQTVFPKGGKTDAAIGTVTTASKSIAAGASADVTSTITAASPKLWSIKNPNLYTVRTEVLNGGKVLDTYDTEYGFRWTGFDATSGFSLNGEKVKLKGVSMHHDQGSLGAVANRRAIERQVEILQKMGVNSIRTTHNPAAKALIDVCNEKGVLVVEEVFDMWNRSKNGNTEDYGKWFGQAIAGDNAVLGGDKDETWAKFDLTSTINRDRNAPSVIMWSLGNEMMEGISGSVSGFPATSAKLVAWTKAADSTRPMTYGDNKIKANWNESNTMGDNLTANGGVVGTNYSDGANYDKIRTTHPSWAIYGSETASAINSRGIYNRTTGGAQSSDKQLTSYDNSAVGWGAVASSAWYDVVQRDFVAGTYVWTGFDYLGEPTPWNGTGSGAVGSWPSPKNSYFGIVDTAGFPKDTYYFYQSQWNDDVHTLHILPAWNENVVAKGSGNNVPVVVYTDAAKVKLYFTPKGSTEKRLIGEKSFTKKTTAAGYTYQVYEGSDKDSTAHKNMYLTWNVPWAEGTISAEAYDENNRLIPEGSTEGNASVTTTGKAAKLKADADRKTITADGKDLSYIEVDVTDANGHIVPDAANRVTFDVKGAGKLVGVDNGSSPDHDSYQADNRKAFSGKVLAIVQSTKEAGEITVTAKADGLQSSTVKIATTAVPGTSTEKTVRSFYYSRNYYVKTGNKPILPSDVEVRYSDGTSDRQNVTWDAVSDDQIAKAGSFSVAGTVAGQKISVRVTMIDEIGALLNYSASTPVGTPAVLPGSRPAVLPDGTVTSANFAVHWTKPADTVYNTAGTVKVPGTATVFGKEFKVTATIRVQRSQVTIGSSVSGNALRLTQNIPADKQSDTLDAIKDGSTTVDANTGGGANPSAWTNWAYSKAGHNTAEITFEYATEQQLGQIVMYFFRDSNAVRFPDAGKTKIQISADGKNWTDLAATETIAAQESSDRVKPYTYDFAPVGATFVKVTVTNADTTTPSGVVCAGLTEIELKTATSKFVTNTSAALSSLTVNGTKVSDSVLAAGSYNTPAIIADVKAEGEGNASVTVLPAHDNVIRVITESEDHVTRKTFTINLGTEQEFPADSDERDYPAADMTVTVGSEQTSGTATEGPKKFAVDGNTSTYWHSNWTPTTVNDLWIAFELQKPTKLDALRYLPRPAGSKNGSVTEYKVQVSDDGTNWTDAGSGTWTTDYGWKLAEFNQPVTTKHVRLKAVHTYADSGNDKFMSASEIRLRKAVDTTDISGATVTVPAKLTVDRVDADHPATFATKDVTVTLGDATLRYGVDYLLDYAGNTAVGKATVTVRGIDKYSGTVAKTFTIELKNAPAPEPTLTSVSVKTKPSKLTYVVGDAFDPAGLVLQLNYDDDSTGTVTWNTQTAGDFTFKPALDAKLKVTDKTVTVTYQGKSAVIDITVSQPAPTVSKTDLDKAIKAIEAKNPDSSKYTADSWKTFADAMAHAKAVIADDSATQQDVDNALKALTDAYAGLTEKTPEPAPVSKSELDKKIKAIEAEKLDGSKYTAESWKAFETALAHAKAVIASDSATQQNVDAALGALTSARDGLTEKGEVKPDPKPEPGTVDKAALDKAVKKVEAEKLDGSKYTADSWKAFETALAHAKAVIGNANSTQFDIDNALSMLNDARAALKEKPGRIIAIIDGSALSKTGASVAIIASVAAAMLAVGAGVMALRRKRS

SEQ ID NO: 2 - protein, 1341 aa, Bifidobacterium bifidum
MKKPLGKIVASTALLISVAFSSSIASAIEDATRSDSTTQMSSTPEVAYSSAVDSKQNRTSDFDANWKFMLSDSVQAQDPAFDDSAWQQVDLPHDYSITQKYSQSNEAESAYLPGGTGWYRKSFTIDRDLAGKRIAINFDGVYMNATVWFNGVKLGTHPYGYSPFSFDLTGNAKFGGENTIVVKVENRLPSSRWYSGSGIYRDVTLTVTDGVHVGNNGVAIKTPSLATQNGGDVTMNLTTKVANDTEAAANITLKQTVFPKGGKTDAAIGTVTTASKSIAAGASADVTSTITAASPKLWSIKNPNLYTVRTEVLNGGKVLDTYDTEYGFRWTGFDATSGFSLNGEKVKLKGVSMHHDQGSLGAVANRRAIERQVEILQKMGVNSIRTTHNPAAKALIDVCNEKGVLVVEEVFDMWNRSKNGNTEDYGKWFGQAIAGDNAVLGGDKDETWAKFDLTSTINRDRNAPSVIMWSLGNEMMEGISGSVSGFSATSAKLVAWTKAADSTRPMTYGDNKIKANWNESNTMGDNLTANGGVVGTNYSDGANYDKIRTTHPSWAIYGSETASAINSRGIYNRTTGGAQSSDKQLTSYDNSAVGWGAVASSAWYDVVQRDFVAGTYVWTGFDYLGEPTPWNGTGSGAVGSWPSPKNSYFGIVDTAGFPKDTYYFYQSQWNDDVHTLHILPAWNENVVAKGSGNNVPVVVYTDAAKVKLYFTPKGSTEQRLIGEKSFTKKTTAAGYTYQVYEGSDKDSTAHKNMYLTWNVPWAEGTISAEAYDENNRLIPEGSTEGNASVTTTGKAAKLKADADRKTITADGKDLSYIEVDVTDANGHIVPDAANRVTFDVKGAGKLVGVDNGSSPDHDSYQADNRKAFSGKVLAIVQSTKEAGEITVTAKADGLQSSTVKIATTAVPGTSTEKTVRSFYYSRNYYVKTGNKPILPSDVEVRYSDGTSDRQNVTWDAVSDDQIAKAGSFSVAGTVAGQKISVRVTMIDEIGALLNYSASTPVGTPAVLPGSRPAVLPDGTVTSANFAVHWTKPADTVYNTAGTVKVPGTATVFGKEFKVTATIRVQRSQVTIGSSVSGNALRLTQNIPADKQSDTLDAIKDGSTTVDANTGGGANPSAWTNWAYSKAGHNTAEITFEYATEQQLGQIVMYFFRDSNAVRFPDAGKTKIQISADGKNWTDLAATETIAAQESSDRVKPYTYDFAPVGATFVRVTVTNADTTTPSGVVCAGLTEIELKTATSKFVANTSAALSSLTVNGTKVSDSVLAAGSYNTPAIIADVKAEGEGNASVTVLPAHDNVIRVITESEDHVTRKTFTINLGTEQEFPADSDERDQHQHQHQHQQ

SEQ ID NO: 3 - protein, 1752 aa, Bifidobacterium bifidum
MAVRRLGGRIVAFAATVALSIPLGLLTNSAWAVEDATRSDSTTQMSSTPEVVYSSAVDSKQNRTSDFDANWKFMLSDSVQAQDPAFDDSAWQQVDLPHDYSITQKYSQSNEAESAYLPGGTGWYRKSFTIDRDLAGKRIAINFDGVYMNATVWFNGVKLGTHPYGYSPFSFDLTGNAKFGGENTIVVKVENRLPSSRWYSGSGIYRDVTLTVTDGVHVGNNGVAIKTPSLATQNGGDVTMNLTTKVANDTEAAANITLKQTVFPKGGKTDAAIGTVTTASKSIAAGASADVTSTITAASPKLWSIKNPNLYTVRTEVLNGGKVLDTYDTEYGFRWTGFDATSGFSLNGEKVKLKGVSMHHDQGSLGAVANRRAIERQVEILQKMGVNSIRTTHNPAAKALIDVCNEKGVLVVEEVFDMWNRSKNGNTEDYGKWFGQAIAGDNAVLGGDKDETWAKFDLTSTINRDRNAPSVIMWSLGNEMMEGISGSVSGFPATSAKLVAWTKAADSTRPMTYGDNKIKANWNESNTMGDNLTANGGVVGTNYSDGANYDKIRTTHPSWAIYGSETASAINSRGIYNRTTGGAQSSDKQLTSYDNSAVGWGAVASSAWYDVVQRDFVAGTYVWTGFDYLGEPTPWNGTGSGAVGSWPSPKNSYFGIVDTAGFPKDTYYFYQSQWNDDVHTLHILPAWNENVVAKGSGNNVPVVVYTDAAKVKLYFTPKGSTEKRLIGEKSFTKKTTAAGYTYQVYEGSDKDSTAHKNMYLTWNVPWAEGTISAEAYDENNRLIPEGSTEGNASVTTTGKAAKLKADADRKTITADGKDLSYIEVDVTDANGHIVPDAANRVTFDVKGAGKLVGVDNGSSPDHDSYQADNRKAFSGKVLAIVQSTKEAGEITVTAKADGLQSSTVKIATTAVPGTSTEKTVRSFYYSRNYYVKTGNKPILPSDVEVRYSDGTSDRQNVTWDAVSDDQIAKAGSFSVAGTVAGQKISVRVTMIDEIGALLNYSASTPVGTPAVLPGSRPAVLPDGTVTSANFAVHWTKPADTVYNTAGTVKVPGTATVFGKEFKVTATIRVQRSQVTIGSSVSGNALRLTQNIPADKQSDTLDAIKDGSTTVDANTGGGANPSAWTNWAYSKAGHNTAEITFEYATEQQLGQIVMYFFRDSNAVRFPDAGKTKIQISADGKNWTDLAATETIAAQESSDRVKPYTYDFAPVGATFVKVTVTNADTTTPSGVVCAGLTEIELKTATSKFVTNTSAALSSLTVNGTKVSDSVLAAGSYNTPAIIADVKAEGEGNASVTVLPAHDNVIRVITESEDHVTRKTFTINLGTEQEFPADSDERDYPAADMTVTVGSEQTSGTATEGPKKFAVDGNTSTYWHSNWTPTTVNDLWIAFELQKPTKLDALRYLPRPAGSKNGSVTEYKVQVSDDGTNWTDAGSGTWTTDYGWKLAEFNQPVTTKHVRLKAVHTYADSGNDKFMSASEIRLRKAVDTTDISGATVTVPAKLTVDRVDADHPATFATKDVTVTLGDATLRYGVDYLLDYAGNTAVGKATVTVRGIDKYSGTVAKTFTIELKNAPAPEPTLTSVSVKTKPSKLTYVVGDAFDPAGLVLQHDRQADRPPQPLVGEQADERGLTCGTRCDRVEQLRKHENREAHRTGLDHLEFVGAADGAVGEQATFKVHVHADQGDGRHDDADERDIDPHVPVDHAVGELARAACHHVIGLRVDTHRLKASGFQIPADDMAEIDRITGFHRFERHVG

SEQ ID NO: 4 - protein, 1935 aa, Bifidobacterium bifidum
MAVRRLGGRIVAFAATVALSIPLGLLTNSAWAVEDATRSDSTTQMSSTPEVVYSSAVDSKQNRTSDFDANWKFMLSDSVQAQDPAFDDSAWQQVDLPHDYSITQKYSQSNEAESAYLPGGTGWYRKSFTIDRDLAGKRIAINFDGVYMNATVWFNGVKLGTHPYGYSPFSFDLTGNAKFGGENTIVVKVENRLPSSRWYSGSGIYRDVTLTVTDGVHVGNNGVAIKTPSLATQNGGNVTMNLTTKVANDTKAAANITLKQTVFPKGGKTDAAIGTVTTASKSIAAGASADVTSTITAASPKLWSIKNPNLYTVRTEVLNGGKVLDTYDTEYGFRWTGFDATSGFSLNGEKVKLKGVSMHHDQGSLGAVANRRAIERQVEILQKMGVNSIRTTHNPAAKALIDVCNEKGVLVVEEVFDMWNRSKNGNTEDYGKWFGQAIAGDNAVLGGDKDETWAKFDLTSTINRDRNAPSVIMWSLGNEMMEGISGSVSGFPATSAKLVAWTKAADSTRPMTYGDNKIKANWNESNTMGDNLTANGGVVGTNYSDGANYDKIRTTHPSWAIYGSETASAINSRGIYNRTTGGAQSSDKQLTSYDNSAVGWGAVASSAWYDVVQRDFVAGTYVWTGFDYLGEPTPWNGTGSGAVGSWPSPKNSYFGIVDTAGFPKDTYYFYQSQWNDDVHTLHILPAWNENVVAKGSGNNVPVVVYTDAAKVKLYFTPKGSTEKRLIGEKSFTKKTTAAGYTYQVYEGADKDSTAHKNMYLTWNVPWAEGTISAEAYDENNRLIPEGSTEGNASVTTTGKAAKLKADADRKTITADGKDLSYIEVDVTDANGHIVPDAANRVTFDVKGAGKLVGVDNGSSPDHDSYQADNRKAFSGKVLAIVQSTKEAGEITVTAKADGLQSSTVKIATTAVPGTSTEKTVRSFYYSRNYYVKTGNKPILPSDVEVRYSDGTSDRQNVTWDAVSDDQIAKAGSFSVAGTVAGQKISVRVTMIDEIGALLNYSASTPVGTPAVLPGSRPAVLPDGTVTSANFAVDWTKPADTVYNTAGTVKVPGTATVFGKEFKVTATIRVQRSQVTIGSSVSGNALRLTQNIPADKQSDTLDAIKDGSTTVDANTGGGANPSAWTNWAYSKAGHNTAEITFEYATEQQLGQIVMYFFRDSNAVRFPDAGKTKIQISADGKNWTDLAATETIAAQESSDRVKPYTYDFAPVGATFVKVTVTNADTTTPSGVVCAGLTEIELKTATSKFVTNTSAALSSLTVNGTKVSDSVLAAGSYNTPAIIADVKAEGEGNASVTVLPAHDNVIRVITESEDHVTRKTFTINLGTEQEFPADSDERDYPAADMTVTAGSEQTSGTATEGPKKFAVDGNTSTYWHSNWTPTTVNDLWIAFELQKPTKLDALRYLPRPAGSKNGSVTEYKVQVSDDGTNWTDAGSGTWTTDYGWKLAEFNQPVTTKHVRLKAVHTYADSGNDKFMSASEIRLRKAVDTTDISGATVTVPAKLTVDRVDADHPATFATKDVTVTLGDATLRYGVDYLLDYAGNTAVGKATVTVRGIDKYSGTVAKTFTIELKNAPAPEPTLTSVSVKTKPSKLTYVVGDAFDPAGLVLQLNYDDDSTGTVTWNTQTAGDFTFKPALDAKLKVTDKTVTVTYQGKSAVIDITVSQPAPTVSKTDLDKAIKAIEAKNPDSSKYTADSWKTFADAMAHAKAVIADDSATQQDVDKALKALTDAYAGLTEKTPEPAPVSKSELDKKIKAIEAEKLDGSKYTAESWKAFETALAHAKAVIASDSATQQDVDAALGALTSARDGLTEKGEVKPDPKPEPGTVDKAALDKAVKKVEAEKLDGSKYTADSWKAFETALAHAKAVIGNANSTQFDIDNALSMLNDARAALKEKPGRIIAIIDGGALSKTGASVAIIASVAAAMKAVGAGVMALRPPKW